European Patent Specification EP 3 858 853 B1, published June 17, 2026. Title: BISPECIFIC CD33 AND CD3 BINDING PROTEINS. Applicant: ELLWANGER, KRISTINA EVNIN, LUKE FOX, JUDITH A. FUCEK, IVICA GUENOT, JEANMARIE KNACKMUSS, STEFAN KUNKEL, LORI LITTLE, MELVYN MOLKENTHIN, VERA RAJKOVIC, ERICH REUSCH, UWE WALL, CLAUDIA WEICHEL, MICHAEL ZHUKOVSKY, EUGENE. Application 14/642,497. The sequence listing filed with the application follows.

SEQUENCE LISTING (122 sequences)

SEQ ID NO: 1 - protein, 108 aa, Homo sapiens
SYELTQPPSVSVAPGQTAMITCGGNNIGSTTVHWYQQKPGQAPVLVVYDDNERPSGIPERFSGSNSGSTATLTINRVEAGDEADYYCQVWDSGSDHVVFGGGTKLTVL

SEQ ID NO: 2 - protein, 110 aa, Homo sapiens
QSVLTQPPSASGTPGQRVTISCSGSRSNIGSNTVNWYQQLPGTAPKLLIYGNNQRPSGVPDRFSGSKSGSSASLAISGLQSEDEADYYCATWDDSLIGWVFGGGTKLTVL

SEQ ID NO: 3 - protein, 110 aa, Homo sapiens
QSVLTQPPSASGTPGQRVTISCSGSRSNIGSNTVNWYQQLPGTAPKLLIYGNNQRPSGVPDRFSGSKSGTSASLAISGLQSEDEADYYCATWDDSLIGWVFGGGTKLTVL

SEQ ID NO: 4 - protein, 110 aa, Homo sapiens; identical to SEQ ID NO: 3

SEQ ID NO: 5 - protein, 110 aa, Homo sapiens; identical to SEQ ID NO: 3

SEQ ID NO: 6 - protein, 110 aa, Homo sapiens
QSVLTQPPSASGTPGQRVTISCSGSSSNIGSNTVNWYQQLPGTAPKLLIYSDNQRPSGVPDRFSGSKSGSSASLAISGLQSDDEADYYCATWDDSLNGAVFGGGTKLTVL

SEQ ID NO: 7 - protein, 111 aa, Homo sapiens
QSVLTQPPSVSGAPGQRVTISCTGSSSNIGAGYDVHWYQQLPGTAPKLLIYGNSNRPSGVPDRFSGSKSGTSASLAITGLQAEDEADYYCQSYDSSLSDVVFGGGTKLTVL

SEQ ID NO: 8 - protein, 110 aa, Homo sapiens
QSVLTQPPSASGTPGQRVTISCSGSSSNIGSNIVNWYQQLPGTAPKLLIYSNNQRPSGVPDRFSGSKSGTSASLAISGLQSEDEADYYCAAWDDSLKGYVFGGGTKLTVL

SEQ ID NO: 9 - protein, 110 aa, Homo sapiens
QSVLTQPPSASGTPGQRVTISCSGSSSNIGSNTVKWYQQLPGTAPKLLIYSNNQRSSGVPDRFSGSKSGSSASLAISGLQSEDEADYYCAAWDDSLNGYVFGGGTKLTVL

SEQ ID NO: 10 - protein, 110 aa, Homo sapiens
QSVLTQPPSASGTPGQRVTISCSGSSSNIGDNVVNWYQQLPGTAPKLLIYSTNKRPSGVPDRFSGSKSGSSASLAISGLQSEDEADYYCAAWDDSLSAYVFGGGTKLTVL

SEQ ID NO: 11 - protein, 119 aa, Homo sapiens
QVQLQESGGGVVQPGRSLRLSCAASGFSFSNYGIHWVRQAPGKGLEWVALISYDGNKKFYADSVKGRFAISRDTSKNTVDLQMTSLRPEDTAVYYCAKDRLESAAFDYWGQGTLVTVSS

SEQ ID NO: 12 - protein, 122 aa, Homo sapiens
QVQLVQSGAEVKKPGASVKVSCKASGYTFTSYDINWVRQAPGQGLEWMGWMNPNSGNTGFAQKFQGRVTMTRDTSTSTVYMELSSLRSEDTAVYYCARDRANTDFSYGMDVWGQGTLVTVSS

SEQ ID NO: 13 - protein, 122 aa, Homo sapiens
QVQLVQSGAEVKKPGASVKVSCKASGYTFTSYDINWVRQAPGQGLEWMGWMNPNSGNTGFAQKFQGRVTMTRDTSTSTVYMELSSLRSEDTAVYYCARDRAVTDYYYGMDVWGQGTLVTVSS

SEQ ID NO: 14 - protein, 122 aa, Homo sapiens
QVQLVQSGAEVKKPGASVKVSCKASGYTFTSYDINWVRQAPGQGLEWMGWMNPNSGNTGFAQKFQGRVTMTRDTSTSTVYMELSSLRSEDTAVYYCARDRANTDYSFGMDVWGQGTLVTVSS

SEQ ID NO: 15 - protein, 122 aa, Homo sapiens
QVQLVQSGAEVKKPGASVKVSCKASGYTFTSYDINWVRQAPGQGLEWMGWMNPNSGNTGFAQKFQGRVTMTRDTSTSTVYMELSSLRSEDTAVYYCARDRANTDYSLGMDVWGQGTLVTVSS

SEQ ID NO: 16 - protein, 123 aa, Homo sapiens
QVQLVQSGAEVKKPGASVKVSCKASGYTFTSYYMHWVRQAPGQGLEWMGIINPSGGSTSYAQKFQGRVTMTRDTSTSTVYMELSSLRSEDTAVYYCARDVVPAAIDYYGMDVWGQGTTVTVSS

SEQ ID NO: 17 - protein, 119 aa, Homo sapiens
QVQLVQSGAEVKKPGESLKISCKGSGYSFTSYWIGWVRQMPGKGLEWMGIIYPGDSDTRYSPSFQGQVTISADKSISTAYLQWSSLKASDTAMYYCARHKRGSDAFDIWGQGTTVTVSS

SEQ ID NO: 18 - protein, 122 aa, Homo sapiens
QVQLVQSGAEVKKPGSSVKVSCKASGGTFSSYAISWVRQAPGQGLEWMGGIYPIFGSANYAQKFQGRVTITADESTSTAYMELSSLRSEDTAVYYCAREYYYDSSEWAFDIWGQGTLVTVSS

SEQ ID NO: 19 - protein, 122 aa, Homo sapiens
QVQLVQSGAEVKKPGSSVKVSCKASGGTFSSYGISWVRQAPGQGLEWMGGIIPIFGSAHYAQKFQGRVTITADESTSTAYMELSSLRSEDTAVYYCAREYYYDSSEWAFDIWGQGTLVTVSS

SEQ ID NO: 20 - protein, 122 aa, Homo sapiens
QVQLVQSGAEVKKPGSSVKVSCKASGGTFDSYAISWVRQAPGQGLEWMGGIIPIFGSAHYSQKFQGRVTITADESTSTAYMELSSLRSEDTAVYYCAREYYYDSSEWAFDIWGQGTLVTVSS

SEQ ID NO: 21 - protein, 11 aa, Homo sapiens
GGNNIGSTTVH

SEQ ID NO: 22 - protein, 13 aa, Homo sapiens
SGSRSNIGSNTVN

SEQ ID NO: 23 - protein, 13 aa, Homo sapiens
SGSSSNIGSNTVN

SEQ ID NO: 24 - protein, 14 aa, Homo sapiens
TGSSSNIGAGYDVH

SEQ ID NO: 25 - protein, 13 aa, Homo sapiens
SGSSSNIGSNIVN

SEQ ID NO: 26 - protein, 13 aa, Homo sapiens
SGSSSNIGSNTVK

SEQ ID NO: 27 - protein, 13 aa, Homo sapiens
SGSSSNIGDNVVN

SEQ ID NO: 28 - protein, 7 aa, Homo sapiens
DDNERPS

SEQ ID NO: 29 - protein, 7 aa, Homo sapiens
GNNQRPS

SEQ ID NO: 30 - protein, 7 aa, Homo sapiens
SDNQRPS

SEQ ID NO: 31 - protein, 7 aa, Homo sapiens
GNSNRPS

SEQ ID NO: 32 - protein, 7 aa, Homo sapiens
SNNQRPS

SEQ ID NO: 33 - protein, 7 aa, Homo sapiens
SNNQRSS

SEQ ID NO: 34 - protein, 7 aa, Homo sapiens
STNKRPS

SEQ ID NO: 35 - protein, 9 aa, Homo sapiens
QVWDSGSDH

SEQ ID NO: 36 - protein, 9 aa, Homo sapiens
ATWDDSLIG

SEQ ID NO: 37 - protein, 9 aa, Homo sapiens
ATWDDSLNG

SEQ ID NO: 38 - protein, 9 aa, Homo sapiens
QSYDSSLSD

SEQ ID NO: 39 - protein, 9 aa, Homo sapiens
AAWDDSLKG

SEQ ID NO: 40 - protein, 9 aa, Homo sapiens
AAWDDSLNG

SEQ ID NO: 41 - protein, 9 aa, Homo sapiens
AAWDDSLSA

SEQ ID NO: 42 - protein, 6 aa, Homo sapiens
SNYGIH

SEQ ID NO: 43 - protein, 6 aa, Homo sapiens
TSYDIN

SEQ ID NO: 44 - protein, 6 aa, Homo sapiens
TSYYMH

SEQ ID NO: 45 - protein, 6 aa, Homo sapiens
TSYWIG

SEQ ID NO: 46 - protein, 6 aa, Homo sapiens
SSYAIS

SEQ ID NO: 47 - protein, 6 aa, Homo sapiens
SSYGIS

SEQ ID NO: 48 - protein, 6 aa, Homo sapiens
DSYAIS

SEQ ID NO: 49 - protein, 17 aa, Homo sapiens
LISYDGNKKFYADSVKG

SEQ ID NO: 50 - protein, 17 aa, Homo sapiens
WMNPNSGNTGFAQKFQG

SEQ ID NO: 51 - protein, 18 aa, Homo sapiens
GIINPSGGSTSYAQKFQG

SEQ ID NO: 52 - protein, 17 aa, Homo sapiens
IIYPGDSDTRYSPSFQG

SEQ ID NO: 53 - protein, 17 aa, Homo sapiens
GIYPIFGSANYAQKFQG

SEQ ID NO: 54 - protein, 17 aa, Homo sapiens
GIIPIFGSAHYAQKFQG

SEQ ID NO: 55 - protein, 17 aa, Homo sapiens
GIIPIFGSAHYSQKFQG

SEQ ID NO: 56 - protein, 10 aa, Homo sapiens
DRLESAAFDY

SEQ ID NO: 57 - protein, 13 aa, Homo sapiens
DRANTDFSYGMDV

SEQ ID NO: 58 - protein, 13 aa, Homo sapiens
DRAVTDYYYGMDV

SEQ ID NO: 59 - protein, 13 aa, Homo sapiens
DRANTDYSFGMDV

SEQ ID NO: 60 - protein, 13 aa, Homo sapiens
DRANTDYSLGMDV

SEQ ID NO: 61 - protein, 14 aa, Homo sapiens
DVVPAAIDYYGMDV

SEQ ID NO: 62 - protein, 10 aa, Homo sapiens
HKRGSDAFDI

SEQ ID NO: 63 - protein, 13 aa, Homo sapiens
EYYYDSSEWAFDI

SEQ ID NO: 64 - protein, 125 aa, Homo sapiens
EVQLVESGGGLVQPGGSLRLSCAASGFTFSTYAMNWVRQAPGKGLEWVGRIRSKYNNYATYYADSVKDRFTISRDDSKNSLYLQMNSLKTEDTAVYYCARHGNFGNSYVSYFAYWGQGTLVTVSS

SEQ ID NO: 65 - protein, 125 aa, Homo sapiens
EVQLVESGGGLVQPGGSLRLSCAASGFTFSTYAMNWVRQAPGKGLEWVGRIRSKYNNYATYYADSVKDRFTISRDDSKNSLYLQMNSLKTEDTAVYYCARHGNFGNSYVSWFAYWGQGTLVTVSS

SEQ ID NO: 66 - protein, 125 aa, Homo sapiens; identical to SEQ ID NO: 65

SEQ ID NO: 67 - protein, 125 aa, Homo sapiens; identical to SEQ ID NO: 65

SEQ ID NO: 68 - protein, 110 aa, Homo sapiens
DIQMTQSPSSLSASVGDRVTITCRSSTGAVTTSNYANWVQQKPGKAPKALIGGTNKRAPGVPSRFSGSLIGDKATLTISSLQPEDFATYYCALWYSNLWVFGQGTKVEIK

SEQ ID NO: 69 - protein, 110 aa, Homo sapiens
DIQMTQSPSSLSASVGDRVTITCRSSTGAVTTSNYANWVQQKPGKAPKGLIGGTNKRAPGVPARFSGSGSGTDFTLTISSLQPEDFATYYCALWYSNLWVFGQGTKVEIK

SEQ ID NO: 70 - protein, 110 aa, Homo sapiens
DIQMTQSPSSLSASVGDRVTITCRSSTGAVTTSNYANWVQQKPGKAPKGLIGGTNKRAPGVPSRFSGSLIGDKATLTISSLQPEDFATYYCALWYSNLWVFGQGTKVEIK

SEQ ID NO: 71 - protein, 110 aa, Homo sapiens
DIQMTQSPSSLSASVGDRVTITCRSSTGAVTTSNYANWVQQKPGKAPKGLIGGTNKRAPGVPSRFSGSLIGTDFTLTISSLQPEDFATYYCALWYSNLWVFGQGTKVEIK

SEQ ID NO: 72 - protein, 6 aa, Homo sapiens
STYAMN

SEQ ID NO: 73 - protein, 19 aa, Homo sapiens
RIRSKYNNYATYYADSVKD

SEQ ID NO: 74 - protein, 14 aa, Homo sapiens
HGNFGNSYVSWFAY

SEQ ID NO: 75 - protein, 14 aa, Homo sapiens
HGNFGNSYVSYFAY

SEQ ID NO: 76 - protein, 6 aa, Homo sapiens
NTYAMN

SEQ ID NO: 77 - protein, 6 aa, Homo sapiens
NTYAMH

SEQ ID NO: 78 - protein, 6 aa, Homo sapiens
NKYAMN

SEQ ID NO: 79 - protein, 19 aa, Homo sapiens
RIRNKYNNYATYYADSVKD

SEQ ID NO: 80 - protein, 19 aa, Homo sapiens
RIRNKYNNYATEYADSVKD

SEQ ID NO: 81 - protein, 19 aa, Homo sapiens
RIRSKYNNYATEYAASVKD

SEQ ID NO: 82 - protein, 19 aa, Homo sapiens
RIRNKYNNYATEYAASVKD

SEQ ID NO: 83 - protein, 19 aa, Homo sapiens
RIRSKYNNYATYYADSVKG

SEQ ID NO: 84 - protein, 19 aa, Homo sapiens
RIRSKYNNYATEYADSVKS

SEQ ID NO: 85 - protein, 14 aa, Homo sapiens
HGNFGDSYVSWFAY

SEQ ID NO: 86 - protein, 14 aa, Homo sapiens
HGNFGNTYVSWFAY

SEQ ID NO: 87 - protein, 14 aa, Homo sapiens
HGNFGCSYVSWFAY

SEQ ID NO: 88 - protein, 14 aa, Homo sapiens
HGNFGNSYISYWAY

SEQ ID NO: 89 - protein, 14 aa, Homo sapiens
HGNFGNSYVSFFAY

SEQ ID NO: 90 - protein, 14 aa, Homo sapiens
RSSTGAVTTSNYAN

SEQ ID NO: 91 - protein, 7 aa, Homo sapiens
GTNKRAP

SEQ ID NO: 92 - protein, 7 aa, Homo sapiens
ALWYSNL

SEQ ID NO: 93 - protein, 242 aa, Homo sapiens
DPNFWLQVQESVTVQEGLCVLVPCTFFHPIPYYDKNSPVHGYWFREGAIISRDSPVATNKLDQEVQEETQGRFRLLGDPSRNNCSLSIVDARRRDNGSYFFRMERGSTKYSYKSPQLSVHVTDLTHRPKILIPGTLEPGHSKNLTCSVSWACEQGTPPIFSWLSAAPTSLGPRTTHSSVLIITPRPQDHGTNLTCQVKFAGAGVTTERTIQLNVTYVPQNPTTGIFPGDGSGKQETRAGVVH

SEQ ID NO: 94 - protein, 9 aa, Homo sapiens
DQEVQEETQ

SEQ ID NO: 95 - protein, 6 aa, Artificial Sequence
  Description of Artificial Sequence: Synthetic peptide
GGSGGS

SEQ ID NO: 96 - protein, 4 aa, Artificial Sequence
  Description of Artificial Sequence: Synthetic peptide
GGSG

SEQ ID NO: 97 - protein, 5 aa, Artificial Sequence
  Description of Artificial Sequence: Synthetic peptide
GGSGG

SEQ ID NO: 98 - protein, 494 aa, Artificial Sequence
  Description of Artificial Sequence: Synthetic polypeptide
DIQMTQSPSSLSASVGDRVTITCRSSTGAVTTSNYANWVQQKPGKAPKGLIGGTNKRAPGVPARFSGSGSGTDFTLTISSLQPEDFATYYCALWYSNLWVFGQGTKVEIKGGSGGSQVQLVQSGAEVKKPGASVKVSCKASGYTFTSYDINWVRQAPGQGLEWMGWMNPNSGNTGFAQKFQGRVTMTRDTSTSTVYMELSSLRSEDTAVYYCARDRANTDFSYGMDVWGQGTLVTVSSGGSGQSVLTQPPSASGTPGQRVTISCSGSRSNIGSNTVNWYQQLPGTAPKLLIYGNNQRPSGVPDRFSGSKSGSSASLAISGLQSEDEADYYCATWDDSLIGWVFGGGTKLTVLGGSGGSEVQLVESGGGLVQPGGSLRLSCAASGFTFSTYAMNWVRQAPGKGLEWVGRIRSKYNNYATYYADSVKDRFTISRDDSKNSLYLQMNSLKTEDTAVYYCARHGNFGNSYVSWFAYWGQGTLVTVSSAAAGSHHHHHH

SEQ ID NO: 99 - protein, 494 aa, Artificial Sequence
  Description of Artificial Sequence: Synthetic polypeptide
DIQMTQSPSSLSASVGDRVTITCRSSTGAVTTSNYANWVQQKPGKAPKGLIGGTNKRAPGVPARFSGSGSGTDFTLTISSLQPEDFATYYCALWYSNLWVFGQGTKVEIKGGSGGSQVQLVQSGAEVKKPGASVKVSCKASGYTFTSYDINWVRQAPGQGLEWMGWMNPNSGNTGFAQKFQGRVTMTRDTSTSTVYMELSSLRSEDTAVYYCARDRAVTDYYYGMDVWGQGTLVTVSSGGSGQSVLTQPPSASGTPGQRVTISCSGSRSNIGSNTVNWYQQLPGTAPKLLIYGNNQRPSGVPDRFSGSKSGTSASLAISGLQSEDEADYYCATWDDSLIGWVFGGGTKLTVLGGSGGSEVQLVESGGGLVQPGGSLRLSCAASGFTFSTYAMNWVRQAPGKGLEWVGRIRSKYNNYATYYADSVKDRFTISRDDSKNSLYLQMNSLKTEDTAVYYCARHGNFGNSYVSWFAYWGQGTLVTVSSAAAGSHHHHHH

SEQ ID NO: 100 - protein, 494 aa, Artificial Sequence
  Description of Artificial Sequence: Synthetic polypeptide
DIQMTQSPSSLSASVGDRVTITCRSSTGAVTTSNYANWVQQKPGKAPKGLIGGTNKRAPGVPARFSGSGSGTDFTLTISSLQPEDFATYYCALWYSNLWVFGQGTKVEIKGGSGGSQVQLVQSGAEVKKPGASVKVSCKASGYTFTSYDINWVRQAPGQGLEWMGWMNPNSGNTGFAQKFQGRVTMTRDTSTSTVYMELSSLRSEDTAVYYCARDRANTDYSFGMDVWGQGTLVTVSSGGSGQSVLTQPPSASGTPGQRVTISCSGSRSNIGSNTVNWYQQLPGTAPKLLIYGNNQRPSGVPDRFSGSKSGTSASLAISGLQSEDEADYYCATWDDSLIGWVFGGGTKLTVLGGSGGSEVQLVESGGGLVQPGGSLRLSCAASGFTFSTYAMNWVRQAPGKGLEWVGRIRSKYNNYATYYADSVKDRFTISRDDSKNSLYLQMNSLKTEDTAVYYCARHGNFGNSYVSWFAYWGQGTLVTVSSAAAGSHHHHHH

SEQ ID NO: 101 - protein, 494 aa, Artificial Sequence
  Description of Artificial Sequence: Synthetic polypeptide
DIQMTQSPSSLSASVGDRVTITCRSSTGAVTTSNYANWVQQKPGKAPKGLIGGTNKRAPGVPARFSGSGSGTDFTLTISSLQPEDFATYYCALWYSNLWVFGQGTKVEIKGGSGGSQVQLVQSGAEVKKPGASVKVSCKASGYTFTSYDINWVRQAPGQGLEWMGWMNPNSGNTGFAQKFQGRVTMTRDTSTSTVYMELSSLRSEDTAVYYCARDRANTDYSLGMDVWGQGTLVTVSSGGSGQSVLTQPPSASGTPGQRVTISCSGSRSNIGSNTVNWYQQLPGTAPKLLIYGNNQRPSGVPDRFSGSKSGTSASLAISGLQSEDEADYYCATWDDSLIGWVFGGGTKLTVLGGSGGSEVQLVESGGGLVQPGGSLRLSCAASGFTFSTYAMNWVRQAPGKGLEWVGRIRSKYNNYATYYADSVKDRFTISRDDSKNSLYLQMNSLKTEDTAVYYCARHGNFGNSYVSWFAYWGQGTLVTVSSAAAGSHHHHHH

SEQ ID NO: 102 - protein, 495 aa, Artificial Sequence
  Description of Artificial Sequence: Synthetic polypeptide
DIQMTQSPSSLSASVGDRVTITCRSSTGAVTTSNYANWVQQKPGKAPKGLIGGTNKRAPGVPARFSGSGSGTDFTLTISSLQPEDFATYYCALWYSNLWVFGQGTKVEIKGGSGGSQVQLVQSGAEVKKPGASVKVSCKASGYTFTSYDINWVRQAPGQGLEWMGWMNPNSGNTGFAQKFQGRVTMTRDTSTSTVYMELSSLRSEDTAVYYCARDRANTDYSFGMDVWGQGTLVTVSSGGSGGQSVLTQPPSASGTPGQRVTISCSGSRSNIGSNTVNWYQQLPGTAPKLLIYGNNQRPSGVPDRFSGSKSGTSASLAISGLQSEDEADYYCATWDDSLIGWVFGGGTKLTVLGGSGGSEVQLVESGGGLVQPGGSLRLSCAASGFTFSTYAMNWVRQAPGKGLEWVGRIRSKYNNYATYYADSVKDRFTISRDDSKNSLYLQMNSLKTEDTAVYYCARHGNFGNSYVSWFAYWGQGTLVTVSSAAAGSHHHHHH

SEQ ID NO: 103 - protein, 495 aa, Artificial Sequence
  Description of Artificial Sequence: Synthetic polypeptide
DIQMTQSPSSLSASVGDRVTITCRSSTGAVTTSNYANWVQQKPGKAPKGLIGGTNKRAPGVPARFSGSGSGTDFTLTISSLQPEDFATYYCALWYSNLWVFGQGTKVEIKGGSGGSQVQLVQSGAEVKKPGASVKVSCKASGYTFTSYDINWVRQAPGQGLEWMGWMNPNSGNTGFAQKFQGRVTMTRDTSTSTVYMELSSLRSEDTAVYYCARDRANTDYSLGMDVWGQGTLVTVSSGGSGGQSVLTQPPSASGTPGQRVTISCSGSRSNIGSNTVNWYQQLPGTAPKLLIYGNNQRPSGVPDRFSGSKSGTSASLAISGLQSEDEADYYCATWDDSLIGWVFGGGTKLTVLGGSGGSEVQLVESGGGLVQPGGSLRLSCAASGFTFSTYAMNWVRQAPGKGLEWVGRIRSKYNNYATYYADSVKDRFTISRDDSKNSLYLQMNSLKTEDTAVYYCARHGNFGNSYVSWFAYWGQGTLVTVSSAAAGSHHHHHH

SEQ ID NO: 104 - protein, 491 aa, Artificial Sequence
  Description of Artificial Sequence: Synthetic polypeptide
DIQMTQSPSSLSASVGDRVTITCRSSTGAVTTSNYANWVQQKPGKAPKALIGGTNKRAPGVPSRFSGSLIGDKATLTISSLQPEDFATYYCALWYSNLWVFGQGTKVEIKGGSGGSQVQLQESGGGVVQPGRSLRLSCAASGFSFSNYGIHWVRQAPGKGLEWVALISYDGNKKFYADSVKGRFAISRDTSKNTVDLQMTSLRPEDTAVYYCAKDRLESAAFDYWGQGTLVTVSSGGSGGSSYELTQPPSVSVAPGQTAMITCGGNNIGSTTVHWYQQKPGQAPVLVVYDDNERPSGIPERFSGSNSGSTATLTINRVEAGDEADYYCQVWDSGSDHVVFGGGTKLTVLGGSGGSEVQLVESGGGLVQPGGSLRLSCAASGFTFSTYAMNWVRQAPGKGLEWVGRIRSKYNNYATYYADSVKDRFTISRDDSKNSLYLQMNSLKTEDTAVYYCARHGNFGNSYVSYFAYWGQGTLVTVSSAAAGSHHHHHH

SEQ ID NO: 105 - protein, 496 aa, Artificial Sequence
  Description of Artificial Sequence: Synthetic polypeptide
QSVLTQPPSASGTPGQRVTISCSGSRSNIGSNTVNWYQQLPGTAPKLLIYGNNQRPSGVPDRFSGSKSGSSASLAISGLQSEDEADYYCATWDDSLIGWVFGGGTKLTVLGGSGGSEVQLVESGGGLVQPGGSLRLSCAASGFTFSTYAMNWVRQAPGKGLEWVGRIRSKYNNYATYYADSVKDRFTISRDDSKNSLYLQMNSLKTEDTAVYYCARHGNFGNSYVSYFAYWGQGTLVTVSSGGSGGSDIQMTQSPSSLSASVGDRVTITCRSSTGAVTTSNYANWVQQKPGKAPKALIGGTNKRAPGVPSRFSGSLIGDKATLTISSLQPEDFATYYCALWYSNLWVFGQGTKVEIKGGSGGSQVQLVQSGAEVKKPGASVKVSCKASGYTFTSYDINWVRQAPGQGLEWMGWMNPNSGNTGFAQKFQGRVTMTRDTSTSTVYMELSSLRSEDTAVYYCARDRANTDFSYGMDVWGQGTLVTVSSAAAGSHHHHHH

SEQ ID NO: 106 - protein, 494 aa, Artificial Sequence
  Description of Artificial Sequence: Synthetic polypeptide
DIQMTQSPSSLSASVGDRVTITCRSSTGAVTTSNYANWVQQKPGKAPKGLIGGTNKRAPGVPSRFSGSLIGDKATLTISSLQPEDFATYYCALWYSNLWVFGQGTKVEIKGGSGGSQVQLVQSGAEVKKPGASVKVSCKASGYTFTSYDINWVRQAPGQGLEWMGWMNPNSGNTGFAQKFQGRVTMTRDTSTSTVYMELSSLRSEDTAVYYCARDRANTDFSYGMDVWGQGTLVTVSSGGSGQSVLTQPPSASGTPGQRVTISCSGSRSNIGSNTVNWYQQLPGTAPKLLIYGNNQRPSGVPDRFSGSKSGSSASLAISGLQSEDEADYYCATWDDSLIGWVFGGGTKLTVLGGSGGSEVQLVESGGGLVQPGGSLRLSCAASGFTFSTYAMNWVRQAPGKGLEWVGRIRSKYNNYATYYADSVKDRFTISRDDSKNSLYLQMNSLKTEDTAVYYCARHGNFGNSYVSWFAYWGQGTLVTVSSAAAGSHHHHHH

SEQ ID NO: 107 - protein, 494 aa, Artificial Sequence
  Description of Artificial Sequence: Synthetic polypeptide
DIQMTQSPSSLSASVGDRVTITCRSSTGAVTTSNYANWVQQKPGKAPKGLIGGTNKRAPGVPSRFSGSLIGDKATLTISSLQPEDFATYYCALWYSNLWVFGQGTKVEIKGGSGGSQVQLVQSGAEVKKPGASVKVSCKASGYTFTSYDINWVRQAPGQGLEWMGWMNPNSGNTGFAQKFQGRVTMTRDTSTSTVYMELSSLRSEDTAVYYCARDRANTDYSFGMDVWGQGTLVTVSSGGSGQSVLTQPPSASGTPGQRVTISCSGSRSNIGSNTVNWYQQLPGTAPKLLIYGNNQRPSGVPDRFSGSKSGTSASLAISGLQSEDEADYYCATWDDSLIGWVFGGGTKLTVLGGSGGSEVQLVESGGGLVQPGGSLRLSCAASGFTFSTYAMNWVRQAPGKGLEWVGRIRSKYNNYATYYADSVKDRFTISRDDSKNSLYLQMNSLKTEDTAVYYCARHGNFGNSYVSWFAYWGQGTLVTVSSAAAGSHHHHHH

SEQ ID NO: 108 - protein, 494 aa, Artificial Sequence
  Description of Artificial Sequence: Synthetic polypeptide
DIQMTQSPSSLSASVGDRVTITCRSSTGAVTTSNYANWVQQKPGKAPKGLIGGTNKRAPGVPSRFSGSLIGDKATLTISSLQPEDFATYYCALWYSNLWVFGQGTKVEIKGGSGGSQVQLVQSGAEVKKPGASVKVSCKASGYTFTSYDINWVRQAPGQGLEWMGWMNPNSGNTGFAQKFQGRVTMTRDTSTSTVYMELSSLRSEDTAVYYCARDRANTDYSLGMDVWGQGTLVTVSSGGSGQSVLTQPPSASGTPGQRVTISCSGSRSNIGSNTVNWYQQLPGTAPKLLIYGNNQRPSGVPDRFSGSKSGTSASLAISGLQSEDEADYYCATWDDSLIGWVFGGGTKLTVLGGSGGSEVQLVESGGGLVQPGGSLRLSCAASGFTFSTYAMNWVRQAPGKGLEWVGRIRSKYNNYATYYADSVKDRFTISRDDSKNSLYLQMNSLKTEDTAVYYCARHGNFGNSYVSWFAYWGQGTLVTVSSAAAGSHHHHHH

SEQ ID NO: 109 - protein, 494 aa, Artificial Sequence
  Description of Artificial Sequence: Synthetic polypeptide
DIQMTQSPSSLSASVGDRVTITCRSSTGAVTTSNYANWVQQKPGKAPKALIGGTNKRAPGVPSRFSGSLIGDKATLTISSLQPEDFATYYCALWYSNLWVFGQGTKVEIKGGSGGSQVQLVQSGAEVKKPGASVKVSCKASGYTFTSYDINWVRQAPGQGLEWMGWMNPNSGNTGFAQKFQGRVTMTRDTSTSTVYMELSSLRSEDTAVYYCARDRAVTDYYYGMDVWGQGTLVTVSSGGSGQSVLTQPPSASGTPGQRVTISCSGSRSNIGSNTVNWYQQLPGTAPKLLIYGNNQRPSGVPDRFSGSKSGTSASLAISGLQSEDEADYYCATWDDSLIGWVFGGGTKLTVLGGSGGSEVQLVESGGGLVQPGGSLRLSCAASGFTFSTYAMNWVRQAPGKGLEWVGRIRSKYNNYATYYADSVKDRFTISRDDSKNSLYLQMNSLKTEDTAVYYCARHGNFGNSYVSYFAYWGQGTLVTVSSAAAGSHHHHHH

SEQ ID NO: 110 - protein, 483 aa, Artificial Sequence
  Description of Artificial Sequence: Synthetic polypeptide
DIQMTQSPSSLSASVGDRVTITCRSSTGAVTTSNYANWVQQKPGKAPKGLIGGTNKRAPGVPSRFSGSLIGTDFTLTISSLQPEDFATYYCALWYSNLWVFGQGTKVEIKGGSGGSQVQLVQSGAEVKKPGASVKVSCKASGYTFTSYDINWVRQAPGQGLEWMGWMNPNSGNTGFAQKFQGRVTMTRDTSTSTVYMELSSLRSEDTAVYYCARDRAVTDYYYGMDVWGQGTLVTVSSGGSGQSVLTQPPSASGTPGQRVTISCSGSRSNIGSNTVNWYQQLPGTAPKLLIYGNNQRPSGVPDRFSGSKSGTSASLAISGLQSEDEADYYCATWDDSLIGWVFGGGTKLTVLGGSGGSEVQLVESGGGLVQPGGSLRLSCAASGFTFSTYAMNWVRQAPGKGLEWVGRIRSKYNNYATYYADSVKDRFTISRDDSKNSLYLQMNSLKTEDTAVYYCARHGNFGNSYVSWFAYWGQGTLVTVSS

SEQ ID NO: 111 - protein, 494 aa, Artificial Sequence
  Description of Artificial Sequence: Synthetic polypeptide
DIQMTQSPSSLSASVGDRVTITCRSSTGAVTTSNYANWVQQKPGKAPKALIGGTNKRAPGVPSRFSGSLIGDKATLTISSLQPEDFATYYCALWYSNLWVFGQGTKVEIKGGSGGSQVQLVQSGAEVKKPGASVKVSCKASGYTFTSYDINWVRQAPGQGLEWMGWMNPNSGNTGFAQKFQGRVTMTRDTSTSTVYMELSSLRSEDTAVYYCARDRANTDFSYGMDVWGQGTLVTVSSGGSGQSVLTQPPSASGTPGQRVTISCSGSRSNIGSNTVNWYQQLPGTAPKLLIYGNNQRPSGVPDRFSGSKSGSSASLAISGLQSEDEADYYCATWDDSLIGWVFGGGTKLTVLGGSGGSEVQLVESGGGLVQPGGSLRLSCAASGFTFSTYAMNWVRQAPGKGLEWVGRIRSKYNNYATYYADSVKDRFTISRDDSKNSLYLQMNSLKTEDTAVYYCARHGNFGNSYVSYFAYWGQGTLVTVSSAAAGSHHHHHH

SEQ ID NO: 112 - protein, 494 aa, Artificial Sequence
  Description of Artificial Sequence: Synthetic polypeptide
DIQMTQSPSSLSASVGDRVTITCRSSTGAVTTSNYANWVQQKPGKAPKALIGGTNKRAPGVPSRFSGSLIGDKATLTISSLQPEDFATYYCALWYSNLWVFGQGTKVEIKGGSGGSQVQLVQSGAEVKKPGASVKVSCKASGYTFTSYDINWVRQAPGQGLEWMGWMNPNSGNTGFAQKFQGRVTMTRDTSTSTVYMELSSLRSEDTAVYYCARDRANTDYSFGMDVWGQGTLVTVSSGGSGQSVLTQPPSASGTPGQRVTISCSGSRSNIGSNTVNWYQQLPGTAPKLLIYGNNQRPSGVPDRFSGSKSGTSASLAISGLQSEDEADYYCATWDDSLIGWVFGGGTKLTVLGGSGGSEVQLVESGGGLVQPGGSLRLSCAASGFTFSTYAMNWVRQAPGKGLEWVGRIRSKYNNYATYYADSVKDRFTISRDDSKNSLYLQMNSLKTEDTAVYYCARHGNFGNSYVSYFAYWGQGTLVTVSSAAAGSHHHHHH

SEQ ID NO: 113 - protein, 494 aa, Artificial Sequence
  Description of Artificial Sequence: Synthetic polypeptide
DIQMTQSPSSLSASVGDRVTITCRSSTGAVTTSNYANWVQQKPGKAPKALIGGTNKRAPGVPSRFSGSLIGDKATLTISSLQPEDFATYYCALWYSNLWVFGQGTKVEIKGGSGGSQVQLVQSGAEVKKPGASVKVSCKASGYTFTSYDINWVRQAPGQGLEWMGWMNPNSGNTGFAQKFQGRVTMTRDTSTSTVYMELSSLRSEDTAVYYCARDRANTDYSLGMDVWGQGTLVTVSSGGSGQSVLTQPPSASGTPGQRVTISCSGSRSNIGSNTVNWYQQLPGTAPKLLIYGNNQRPSGVPDRFSGSKSGTSASLAISGLQSEDEADYYCATWDDSLIGWVFGGGTKLTVLGGSGGSEVQLVESGGGLVQPGGSLRLSCAASGFTFSTYAMNWVRQAPGKGLEWVGRIRSKYNNYATYYADSVKDRFTISRDDSKNSLYLQMNSLKTEDTAVYYCARHGNFGNSYVSYFAYWGQGTLVTVSSAAAGSHHHHHH

SEQ ID NO: 114 - protein, 492 aa, Artificial Sequence
  Description of Artificial Sequence: Synthetic polypeptide
DIQMTQSPSSLSASVGDRVTITCRSSTGAVTTSNYANWVQQKPGKAPKALIGGTNKRAPGVPSRFSGSLIGDKATLTISSLQPEDFATYYCALWYSNLWVFGQGTKVEIKGGSGGSQVQLVQSGAEVKKPGESLKISCKGSGYSFTSYWIGWVRQMPGKGLEWMGIIYPGDSDTRYSPSFQGQVTISADKSISTAYLQWSSLKASDTAMYYCARHKRGSDAFDIWGQGTTVTVSSGGSGQSVLTQPPSVSGAPGQRVTISCTGSSSNIGAGYDVHWYQQLPGTAPKLLIYGNSNRPSGVPDRFSGSKSGTSASLAITGLQAEDEADYYCQSYDSSLSDVVFGGGTKLTVLGGSGGSEVQLVESGGGLVQPGGSLRLSCAASGFTFSTYAMNWVRQAPGKGLEWVGRIRSKYNNYATYYADSVKDRFTISRDDSKNSLYLQMNSLKTEDTAVYYCARHGNFGNSYVSYFAYWGQGTLVTVSSAAAGSHHHHHH

SEQ ID NO: 115 - protein, 492 aa, Artificial Sequence
  Description of Artificial Sequence: Synthetic polypeptide
EVQLVESGGGLVQPGGSLRLSCAASGFTFSTYAMNWVRQAPGKGLEWVGRIRSKYNNYATYYADSVKDRFTISRDDSKNSLYLQMNSLKTEDTAVYYCARHGNFGNSYVSYFAYWGQGTLVTVSSGGSGGSQSVLTQPPSVSGAPGQRVTISCTGSSSNIGAGYDVHWYQQLPGTAPKLLIYGNSNRPSGVPDRFSGSKSGTSASLAITGLQAEDEADYYCQSYDSSLSDVVFGGGTKLTVLGGSGQVQLVQSGAEVKKPGESLKISCKGSGYSFTSYWIGWVRQMPGKGLEWMGIIYPGDSDTRYSPSFQGQVTISADKSISTAYLQWSSLKASDTAMYYCARHKRGSDAFDIWGQGTTVTVSSGGSGGSDIQMTQSPSSLSASVGDRVTITCRSSTGAVTTSNYANWVQQKPGKAPKALIGGTNKRAPGVPSRFSGSLIGDKATLTISSLQPEDFATYYCALWYSNLWVFGQGTKVEIKAAAGSHHHHHH

SEQ ID NO: 116 - protein, 495 aa, Artificial Sequence
  Description of Artificial Sequence: Synthetic polypeptide
DIQMTQSPSSLSASVGDRVTITCRSSTGAVTTSNYANWVQQKPGKAPKALIGGTNKRAPGVPSRFSGSLIGDKATLTISSLQPEDFATYYCALWYSNLWVFGQGTKVEIKGGSGGSQVQLVQSGAEVKKPGASVKVSCKASGYTFTSYYMHWVRQAPGQGLEWMGIINPSGGSTSYAQKFQGRVTMTRDTSTSTVYMELSSLRSEDTAVYYCARDVVPAAIDYYGMDVWGQGTTVTVSSGGSGQSVLTQPPSASGTPGQRVTISCSGSSSNIGSNTVNWYQQLPGTAPKLLIYSDNQRPSGVPDRFSGSKSGSSASLAISGLQSDDEADYYCATWDDSLNGAVFGGGTKLTVLGGSGGSEVQLVESGGGLVQPGGSLRLSCAASGFTFSTYAMNWVRQAPGKGLEWVGRIRSKYNNYATYYADSVKDRFTISRDDSKNSLYLQMNSLKTEDTAVYYCARHGNFGNSYVSYFAYWGQGTLVTVSSAAAGSHHHHHH

SEQ ID NO: 117 - protein, 484 aa, Artificial Sequence
  Description of Artificial Sequence: Synthetic polypeptide
DIQMTQSPSSLSASVGDRVTITCRSSTGAVTTSNYANWVQQKPGKAPKGLIGGTNKRAPGVPSRFSGSLIGTDFTLTISSLQPEDFATYYCALWYSNLWVFGQGTKVEIKGGSGGSQVQLVQSGAEVKKPGASVKVSCKASGYTFTSYYMHWVRQAPGQGLEWMGIINPSGGSTSYAQKFQGRVTMTRDTSTSTVYMELSSLRSEDTAVYYCARDVVPAAIDYYGMDVWGQGTTVTVSSGGSGQSVLTQPPSASGTPGQRVTISCSGSSSNIGSNTVNWYQQLPGTAPKLLIYSDNQRPSGVPDRFSGSKSGSSASLAISGLQSDDEADYYCATWDDSLNGAVFGGGTKLTVLGGSGGSEVQLVESGGGLVQPGGSLRLSCAASGFTFSTYAMNWVRQAPGKGLEWVGRIRSKYNNYATYYADSVKDRFTISRDDSKNSLYLQMNSLKTEDTAVYYCARHGNFGNSYVSWFAYWGQGTLVTVSS

SEQ ID NO: 118 - protein, 494 aa, Artificial Sequence
  Description of Artificial Sequence: Synthetic polypeptide
DIQMTQSPSSLSASVGDRVTITCRSSTGAVTTSNYANWVQQKPGKAPKALIGGTNKRAPGVPSRFSGSLIGDKATLTISSLQPEDFATYYCALWYSNLWVFGQGTKVEIKGGSGGSQVQLVQSGAEVKKPGSSVKVSCKASGGTFSSYAISWVRQAPGQGLEWMGGIYPIFGSANYAQKFQGRVTITADESTSTAYMELSSLRSEDTAVYYCAREYYYDSSEWAFDIWGQGTLVTVSSGGSGQSVLTQPPSASGTPGQRVTISCSGSSSNIGSNIVNWYQQLPGTAPKLLIYSNNQRPSGVPDRFSGSKSGTSASLAISGLQSEDEADYYCAAWDDSLKGYVFGGGTKLTVLGGSGGSEVQLVESGGGLVQPGGSLRLSCAASGFTFSTYAMNWVRQAPGKGLEWVGRIRSKYNNYATYYADSVKDRFTISRDDSKNSLYLQMNSLKTEDTAVYYCARHGNFGNSYVSYFAYWGQGTLVTVSSAAAGSHHHHHH

SEQ ID NO: 119 - protein, 494 aa, Artificial Sequence
  Description of Artificial Sequence: Synthetic polypeptide
DIQMTQSPSSLSASVGDRVTITCRSSTGAVTTSNYANWVQQKPGKAPKALIGGTNKRAPGVPSRFSGSLIGDKATLTISSLQPEDFATYYCALWYSNLWVFGQGTKVEIKGGSGGSQVQLVQSGAEVKKPGSSVKVSCKASGGTFSSYGISWVRQAPGQGLEWMGGIIPIFGSAHYAQKFQGRVTITADESTSTAYMELSSLRSEDTAVYYCAREYYYDSSEWAFDIWGQGTLVTVSSGGSGQSVLTQPPSASGTPGQRVTISCSGSSSNIGSNTVKWYQQLPGTAPKLLIYSNNQRSSGVPDRFSGSKSGSSASLAISGLQSEDEADYYCAAWDDSLNGYVFGGGTKLTVLGGSGGSEVQLVESGGGLVQPGGSLRLSCAASGFTFSTYAMNWVRQAPGKGLEWVGRIRSKYNNYATYYADSVKDRFTISRDDSKNSLYLQMNSLKTEDTAVYYCARHGNFGNSYVSYFAYWGQGTLVTVSSAAAGSHHHHHH

SEQ ID NO: 120 - protein, 483 aa, Artificial Sequence
  Description of Artificial Sequence: Synthetic polypeptide
DIQMTQSPSSLSASVGDRVTITCRSSTGAVTTSNYANWVQQKPGKAPKGLIGGTNKRAPGVPSRFSGSLIGTDFTLTISSLQPEDFATYYCALWYSNLWVFGQGTKVEIKGGSGGSQVQLVQSGAEVKKPGSSVKVSCKASGGTFSSYGISWVRQAPGQGLEWMGGIIPIFGSAHYAQKFQGRVTITADESTSTAYMELSSLRSEDTAVYYCAREYYYDSSEWAFDIWGQGTLVTVSSGGSGQSVLTQPPSASGTPGQRVTISCSGSSSNIGSNTVKWYQQLPGTAPKLLIYSNNQRSSGVPDRFSGSKSGSSASLAISGLQSEDEADYYCAAWDDSLNGYVFGGGTKLTVLGGSGGSEVQLVESGGGLVQPGGSLRLSCAASGFTFSTYAMNWVRQAPGKGLEWVGRIRSKYNNYATYYADSVKDRFTISRDDSKNSLYLQMNSLKTEDTAVYYCARHGNFGNSYVSWFAYWGQGTLVTVSS

SEQ ID NO: 121 - protein, 494 aa, Artificial Sequence
  Description of Artificial Sequence: Synthetic polypeptide
DIQMTQSPSSLSASVGDRVTITCRSSTGAVTTSNYANWVQQKPGKAPKALIGGTNKRAPGVPSRFSGSLIGDKATLTISSLQPEDFATYYCALWYSNLWVFGQGTKVEIKGGSGGSQVQLVQSGAEVKKPGSSVKVSCKASGGTFDSYAISWVRQAPGQGLEWMGGIIPIFGSAHYSQKFQGRVTITADESTSTAYMELSSLRSEDTAVYYCAREYYYDSSEWAFDIWGQGTLVTVSSGGSGQSVLTQPPSASGTPGQRVTISCSGSSSNIGDNVVNWYQQLPGTAPKLLIYSTNKRPSGVPDRFSGSKSGSSASLAISGLQSEDEADYYCAAWDDSLSAYVFGGGTKLTVLGGSGGSEVQLVESGGGLVQPGGSLRLSCAASGFTFSTYAMNWVRQAPGKGLEWVGRIRSKYNNYATYYADSVKDRFTISRDDSKNSLYLQMNSLKTEDTAVYYCARHGNFGNSYVSYFAYWGQGTLVTVSSAAAGSHHHHHH

SEQ ID NO: 122 - protein, 6 aa, Artificial Sequence
  Description of Artificial Sequence: Synthetic 6xHis tag
HHHHHH